European Patent Specification EP 3 391 880 B1, published June 7, 2023. Title: USE OF NEDDYLATION INHIBITOR FOR PREVENTING OR TREATING OSTEOPOROSIS. Applicant: Chang Gung University Chiayi Chang Gung Memorial Hospital. The sequence listing filed with the application follows.

SEQUENCE LISTING (8 sequences)

SEQ ID NO: 1 - DNA, 21 bp, Artificial Sequence
  synthesized
ggagccaauggcuguugautt

SEQ ID NO: 2 - DNA, 21 bp, Artificial Sequence
  synthesized
ttccucgguuaccgacaacua

SEQ ID NO: 3 - DNA, 21 bp, Artificial Sequence
  synthesized
ggaucaauggaaugcugautt

SEQ ID NO: 4 - DNA, 21 bp, Artificial Sequence
  synthesized
ttccuaguuaccuuacgacua

SEQ ID NO: 5 - DNA, 21 bp, Artificial Sequence
  synthesized
ccaagcuccauuguaccuutt

SEQ ID NO: 6 - DNA, 21 bp, Artificial Sequence
  synthesized
ttgguucgagguaacauggaa

SEQ ID NO: 7 - DNA, 21 bp, Artificial Sequence
  synthesized
uucuccgaacgugucacgutt

SEQ ID NO: 8 - DNA, 21 bp, Artificial Sequence
  synthesized
ttaagaggcuugcacagugca